European Patent Application EP 4 721 765 A1, published April 8, 2026. Title: BI-FUNCTIONALIZED ANTIBODY CONJUGATES AGAINST THE ENDOTHELIN RECEPTOR B. Applicant: COMMISSARIAT A l'ENERGIE ATOMIQUE ET AUX ENERGIES ALTERNATIVES. Application EP. The sequence listing filed with the application follows.

SEQUENCE LISTING (27 sequences)

SEQ ID NO: 1 - protein, 11 aa, mus musculus
  REGION 1..11: note = MISC_FEATURE - LCDR1 of Rendomab B4
QSLLDSDGKTY

SEQ ID NO: 2 - skipped

SEQ ID NO: 3 - protein, 9 aa, mus musculus
  REGION 1..9: note = MISC_FEATURE - LCDR3 of Rendomab B4
WQGTHFPQT

SEQ ID NO: 4 - protein, 8 aa, mus musculus
  REGION 1..8: note = MISC_FEATURE - HCDR1 of Rendomab B4
GYTFTDYT

SEQ ID NO: 5 - protein, 8 aa, mus musculus
  REGION 1..8: note = MISC_FEATURE - HCDR2 of Rendomab B4
FYPGSDNI

SEQ ID NO: 6 - protein, 12 aa, mus musculus
  REGION 1..12: note = MISC_FEATURE - HCDR3 of Rendomab B4
ARLVFFTGALDY

SEQ ID NO: 7 - protein, 112 aa, mus musculus
  REGION 1..112: note = MISC_FEATURE - Light Chain variable domain of Rendomab B4
DIVMTQTPLTLSVIIGQPASISCKSSQSLLDSDGKTYLNWLLQRPGQAPKRLIYLVSKLDSGVPDRFTGSGSGTDFTLKISRVEAEDLGVYYCWQGTHFPQTFGGGTKLEIK

SEQ ID NO: 8 - protein, 119 aa, mus musculus
  REGION 1..119: note = MISC_FEATURE - Heavy Chain variable domain of Rendomab B4
QVQLQQSGAELVKPGASVKLSCKASGYTFTDYTIHWVKQRSGQGLEWIGWFYPGSDNIKYSERFKDKATLTADKSSSTVYMELSRLTSEDSAVYFCARLVFFTGALDYWGQGTSVTVSS

SEQ ID NO: 9 - protein, 11 aa, homo sapiens
  REGION 1..11: note = MISC_FEATURE - epitope of human ETB recognized by Rendomab B4
ERGFPPDRATP

SEQ ID NO: 10 - protein, 8 aa, homo sapiens
  REGION 1..8: note = MISC_FEATURE - epitope of human ETB recognized by Rendomab B4
EVPKGDRT

SEQ ID NO: 11 - protein, 442 aa, homo sapiens
  REGION 1..442: note = MISC_FEATURE - P24530
MQPPPSLCGRALVALVLACGLSRIWGEERGFPPDRATPLLQTAEIMTPPTKTLWPKGSNASLARSLAPAEVPKGDRTAGSPPRTISPPPCQGPIEIKETFKYINTVVSCLVFVLGIIGNSTLLRIIYKNKCMRNGPNILIASLALGDLLHIVIDIPINVYKLLAEDWPFGAEMCKLVPFIQKASVGITVLSLCALSIDRYRAVASWSRIKGIGVPKWTAVEIVLIWVVSVVLAVPEAIGFDIITMDYKGSYLRICLLHPVQKTAFMQFYKTAKDWWLFSFYFCLPLAITAFFYTLMTCEMLRKKSGMQIALNDHLKQRREVAKTVFCLVLVFALCWLPLHLSRILKLTLYNQNDPNRCELLSFLLVLDYIGINMASLNSCINPIALYLVSKRFKNCFKSCLCCWCQSFEEKQSLEEKQSCLKFKANDHGYDNFRSSNKYSSS

SEQ ID NO: 12 - DNA, 33 bp, synthetic construct
  misc_feature 1..33: note = polynucleotide sequence encoding CDR1 of the light chain of Rendomab B4
  source 1..33: mol_type = other DNA
cagagcctcttagatagtgatggaaagacatat

SEQ ID NO: 13 - skipped

SEQ ID NO: 14 - DNA, 27 bp, synthetic construct
  misc_feature 1..27: note = polynucleotide encoding the CDR3 of the light chain of Rendomab B4
  source 1..27: mol_type = other DNA
tggcaaggtacacattttcctcagacg

SEQ ID NO: 15 - DNA, 336 bp, synthetic construct
  misc_feature 1..336: note = polynucleotide encoding the light variable chain of Rendomab B4
  source 1..336: mol_type = other DNA
gatatagtgatgacccagactccactcactttgtcggttatcattggacaaccagcctccatctcttgcaagtcaagtcagagcctcttagatagtgatggaaagacatatttgaattggttgttacagaggccaggccaggctccaaagcgcctaatctatctggtgtctaaactggactctggagtccctgacaggttcactggcagtggatcagggacagatttcacactgaaaatcagcagagtggaggctgaggatttgggagtttattattgctggcaaggtacacattttcctcagacgttcggtggaggcaccaagctggaaatcaaa

SEQ ID NO: 16 - DNA, 24 bp, synthetic construct
  misc_feature 1..24: note = polynucleotide encoding the CDR1 of the heavy chain of Rendomab B4
  source 1..24: mol_type = other DNA
ggctacaccttcactgactatact

SEQ ID NO: 17 - DNA, 24 bp, synthetic construct
  misc_feature 1..24: note = polynucleotide encoding the CDR2 of the heavy chain of Rendomab B4
  source 1..24: mol_type = other DNA
ttttaccctggaagtgataatata

SEQ ID NO: 18 - DNA, 36 bp, synthetic construct
  misc_feature 1..36: note = polynucleotide encoding the CDR3 of the heavy chain of Rendomab B4
  source 1..36: mol_type = other DNA
gcaagactcgtattttttactggggctttggactac

SEQ ID NO: 19 - DNA, 357 bp, synthetic construct
  misc_feature 1..357: note = polynucleotide encoding the heavy variable chain of Rendomab B4
  source 1..357: mol_type = other DNA
caggtccagctgcagcagtctggagctgagctggtgaaacccggggcatcagtgaagctgtcctgcaaggcttctggctacaccttcactgactatactatacactgggtaaagcagaggtctggacagggtcttgagtggattgggtggttttaccctggaagtgataatataaagtacagtgagagattcaaggacaaggccacattgactgcggacaaatcctccagcacagtctatatggagcttagtagattgacatctgaagactctgcggtctatttctgtgcaagactcgtattttttactggggctttggactactggggtcaaggaacctcagtcaccgtctcctca

SEQ ID NO: 20 - DNA, 27 bp, synthetic construct
  misc_feature 1..27: note = forward primer for amplification of rat ETB
  source 1..27: mol_type = other DNA
gcaagcttatgcaatcgtccgcaagcc

SEQ ID NO: 21 - DNA, 33 bp, synthetic construct
  misc_feature 1..33: note = Reverse primer for amplification of rat ETB
  source 1..33: mol_type = other DNA
gcggatccacagatgagctgtatttattgctgg

SEQ ID NO: 22 - protein, 219 aa, synthetic construct
DIVMTQTPLTLSVIIGQPASISCKSSQSLLDSDGKTYLNWLLQRPGQAPKRLIYLVSKLDSGVPDRFTGSGSGTDFTLKISRVEAEDLGVYYCWQGTHFPQTFGGGTKLEIKRTVAAPSVFIFPPSDEQLKSGTASVVCLLNNFYPREAKVQWKVDNALQSGNSQESVTEQDSKDSTYSLSSTLTLSKADYEKHKVYACEVTHQGLSSPVTKSFNRGEC

SEQ ID NO: 23 - protein, 449 aa, synthetic construct
QVQLQQSGAELVKPGASVKLSCKASGYTFTDYTIHWVKQRSGQGLEWIGWFYPGSDNIKYSERFKDKATLTADKSSSTVYMELSRLTSEDSAVYFCARLVFFTGALDYWGQGTSVTVSSASTKGPSVFPLAPSSKSTSGGTAALGCLVKDYFPEPVTVSWNSGALTSGVHTFPAVLQSSGLYSLSSVVTVPSSSLGTQTYICNVNHKPSNTKVDKKVEPKSCDKTHTCPPCPAPELLGGPSVFLFPPKPKDTLMISRTPEVTCVVVDVSHEDPEVKFNWYVDGVEVHNAKTKPREEQYNSTYRVVSVLTVLHQDWLNGKEYKCKVSNKALPAPIEKTISKAKGQPREPQVYTLPPSREEMTKNQVSLTCLVKGFYPSDIAVEWESNGQPENNYKTTPPVLDSDGSFFLYSKLTVDKSRWQQGNVFSCSVMHEALHNHYTQKSLSLSPGK

SEQ ID NO: 24 - protein, 219 aa, synthetic construct; identical to SEQ ID NO: 22

SEQ ID NO: 25 - protein, 226 aa, synthetic construct
QVQLQQSGAELVKPGASVKLSCKASGYTFTDYTIHWVKQRSGQGLEWIGWFYPGSDNIKYSERFKDKATLTADKSSSTVYMELSRLTSEDSAVYFCARLVFFTGALDYWGQGTSVTVSSASTKGPSVFPLAPSSKSTSGGTAALGCLVKDYFPEPVTVSWNSGALTSGVHTFPAVLQSSGLYSLSSVVTVPSSSLGTQTYICNVNHKPSNTKVDKKVEPKSCDKTH

SEQ ID NO: 26 - protein, 224 aa, synthetic construct
DIVMTQTPLTLSVIIGQPASISCKSSQSLLDSDGKTYLNWLLQRPGQAPKRLIYLVSKLDSGVPDRFTGSGSGTDFTLKISRVEAEDLGVYYCWQGTHFPQTFGGGTKLEIKRTVAAPSVFIFPPSDEQLKSGTASVVCLLNNFYPREAKVQWKVDNALQSGNSQESVTEQDSKDSTYSLSSTLTLSKADYEKHKVYACEVTHQGLSSPVTKSFNRGECLLQGA

SEQ ID NO: 27 - protein, 5 aa, synthetic construct
LLQGA